European Patent Specification EP 3 686 601 B1, published May 10, 2023. Title: Serological detection of Plasmodium antibodies. Applicant: EUROIMMUN Medizinische Labordiagnostika AG. The sequence listing filed with the application follows.

SEQUENCE LISTING (34 sequences)

SEQ ID NO: 1 - protein, 61 aa, Artificial Sequence
  Plasmodium p19 consensus motif; Xaa at position 4, 35, 50 and 54 stands for at least one amino acid; Glu at position 6 can also be Asp; Asp at position 56 can also be Glu.
  misc_feature (2)..(2): Xaa can be any naturally occurring amino acid
  misc_feature (4)..(4): Xaa can be any naturally occurring amino acid
  misc_feature (8)..(9): Xaa can be any naturally occurring amino acid
  misc_feature (11)..(11): Xaa can be any naturally occurring amino acid
  misc_feature (13)..(14): Xaa can be any naturally occurring amino acid
  misc_feature (16)..(17): Xaa can be any naturally occurring amino acid
  misc_feature (19)..(21): Xaa can be any naturally occurring amino acid
  misc_feature (25)..(26): Xaa can be any naturally occurring amino acid
  misc_feature (28)..(32): Xaa can be any naturally occurring amino acid
  misc_feature (35)..(35): Xaa can be any naturally occurring amino acid
  misc_feature (37)..(38): Xaa can be any naturally occurring amino acid
  misc_feature (44)..(46): Xaa can be any naturally occurring amino acid
  misc_feature (48)..(48): Xaa can be any naturally occurring amino acid
  misc_feature (50)..(50): Xaa can be any naturally occurring amino acid
  misc_feature (52)..(52): Xaa can be any naturally occurring amino acid
  misc_feature (54)..(54): Xaa can be any naturally occurring amino acid
  misc_feature (58)..(58): Xaa can be any naturally occurring amino acid
  misc_feature (61)..(61): Xaa can be any naturally occurring amino acid
HXCXPENXXCXRXXDXXEXXXCLLXXKXXXXXCVXCXXNNGGCXXXAXCXCXCXFDGXFCX

SEQ ID NO: 2 - protein, 93 aa, Plasmodium falciparum
NISQHQCVKKQCPENSGCFRHLDEREECKCLLNYKQEGDKCVENPNPTCNENNGGCDADAKCTEEDSGSNGKKITCECTKPDSYPLFDGIFCS

SEQ ID NO: 3 - protein, 90 aa, Plasmodium vivax
TMSSEHTCIDTNVPDNAACYRYLDGTEEWRCLLTFKEEGGKCVPASNVTCKDNNGGCAPEAECKMTDSNKIVCKCTKEGSEPLFEGVFCS

SEQ ID NO: 4 - protein, 89 aa, Plasmodium ovale
SMGSKHKCIDITYPDNAGCYRFSDGREEWRCLLNFKKVGETCVPNNNPTCAENNGGCDPTADCAESENNKITCTCTGQNESFFEGVFCG

SEQ ID NO: 5 - protein, 90 aa, Plasmodium malariae
NISAKHACTETKYPENAGCYRYEDGKEVWRCLLNYKLVDGGCVEDEEPSCQVNNGGCAPEANCTKGDDNKIVCACNAPYSEPIFEGVFCG

SEQ ID NO: 6 - protein, 89 aa, Plasmodium knowlesi
NMSSAHKCIDTNVPENAACYRYLDGTEEWRCLLGFKEVGGKCVPASITCEENNGGCAPEAECTMDDKKEVECKCTKEGFEPLFEGVFCS

SEQ ID NO: 7 - protein, 200 aa, Artificial Sequence
  Plasmodium p33 consensus motif; Xaa at position 118 and at position 181 stands for at least one amino acid
  misc_feature (2)..(2): Xaa can be any naturally occurring amino acid
  misc_feature (4)..(4): Xaa can be any naturally occurring amino acid
  misc_feature (6)..(6): Xaa can be any naturally occurring amino acid
  misc_feature (12)..(12): Xaa can be any naturally occurring amino acid
  misc_feature (14)..(17): Xaa can be any naturally occurring amino acid
  misc_feature (20)..(26): Xaa can be any naturally occurring amino acid
  misc_feature (28)..(29): Xaa can be any naturally occurring amino acid
  misc_feature (31)..(34): Xaa can be any naturally occurring amino acid
  misc_feature (36)..(37): Xaa can be any naturally occurring amino acid
  misc_feature (39)..(39): Xaa can be any naturally occurring amino acid
  misc_feature (43)..(43): Xaa can be any naturally occurring amino acid
  misc_feature (47)..(47): Xaa can be any naturally occurring amino acid
  misc_feature (50)..(50): Xaa can be any naturally occurring amino acid
  misc_feature (52)..(52): Xaa can be any naturally occurring amino acid
  misc_feature (54)..(56): Xaa can be any naturally occurring amino acid
  misc_feature (58)..(60): Xaa can be any naturally occurring amino acid
  misc_feature (62)..(63): Xaa can be any naturally occurring amino acid
  misc_feature (65)..(65): Xaa can be any naturally occurring amino acid
  misc_feature (67)..(67): Xaa can be any naturally occurring amino acid
  misc_feature (69)..(70): Xaa can be any naturally occurring amino acid
  misc_feature (74)..(77): Xaa can be any naturally occurring amino acid
  misc_feature (79)..(80): Xaa can be any naturally occurring amino acid
  misc_feature (82)..(83): Xaa can be any naturally occurring amino acid
  misc_feature (86)..(86): Xaa can be any naturally occurring amino acid
  misc_feature (89)..(94): Xaa can be any naturally occurring amino acid
  misc_feature (96)..(98): Xaa can be any naturally occurring amino acid
  misc_feature (100)..(101): Xaa can be any naturally occurring amino acid
  misc_feature (103)..(104): Xaa can be any naturally occurring amino acid
  misc_feature (107)..(107): Xaa can be any naturally occurring amino acid
  misc_feature (109)..(112): Xaa can be any naturally occurring amino acid
  misc_feature (115)..(116): Xaa can be any naturally occurring amino acid
  misc_feature (118)..(118): Xaa can be any naturally occurring amino acid
  misc_feature (120)..(121): Xaa can be any naturally occurring amino acid
  misc_feature (125)..(130): Xaa can be any naturally occurring amino acid
  misc_feature (132)..(133): Xaa can be any naturally occurring amino acid
  misc_feature (135)..(144): Xaa can be any naturally occurring amino acid
  misc_feature (147)..(151): Xaa can be any naturally occurring amino acid
  misc_feature (153)..(154): Xaa can be any naturally occurring amino acid
  misc_feature (157)..(164): Xaa can be any naturally occurring amino acid
  misc_feature (167)..(172): Xaa can be any naturally occurring amino acid
  misc_feature (174)..(179): Xaa can be any naturally occurring amino acid
  misc_feature (181)..(181): Xaa can be any naturally occurring amino acid
  misc_feature (183)..(197): Xaa can be any naturally occurring amino acid
  misc_feature (199)..(199): Xaa can be any naturally occurring amino acid
YXVXYXKPLAGXYXXXXKQXXXXXXXFXXNXXXXLXXRXKKRXYFLXVLXSXLXXXKXXXSXXYXIXDXXKLLXXXXKXXLXXSYXYIXXXXXXDXXXAXXGXXYYXKXXXXYKXXLXKXXPFLXXXXXXYXXLXXXXXXXXXXLKXXXXXCXXEKXXXXXXXXKLXXXXXXDXXXXXXKXLXXXXXXXXXXXXXXXSXL

SEQ ID NO: 8 - protein, 280 aa, Plasmodium falciparum
AISVTMDNILSGFENEYDVIYLKPLAGVYRSLKKQIEKNIFTFNLNLNDILNSRLKKRKYFLDVLESDLMQFKHISSNEYIIEDSFKLLNSEQKNTLLKSYKYIKESVENDIKFAQEGISYYEKVLAKYKDDLESIKKVIKEEKEKFPSSPPTTPPSPAKTDEQKKESKFLPFLTNIETLYNNLVNKIDDYLINLKAKINDCNVEKDEAHVKITKLSDLKAIDDKIDLFKNPYDFEAIKKLINDDTKKDMLGKLLSTGLVQNFPNTIISKLIEGKFQDML

SEQ ID NO: 9 - protein, 290 aa, Plasmodium vivax
DQVTTGEAESEAPEILVPAGISDYDVVYLKPLAGMYKTIKKQLENHVNAFNTNITDMLDSRLKKRNYFLEVLNSDLNPFKYSSSGEYIIKDPYKLLDLEKKKKLIGSYKYIGASIDMDLATANDGVTYYNKMGELYKTHLDGVKTEIKKVEDDIKKQDEELKKLGNVNSQDSKKNEFIAKKAELEKYLPFLNSLQKEYESLVSKVNTYTDNLKKVINNCQLEKKEAEITVKKLQDYNKMDEKLEEYKKSEKKNEVKSSGLLEKLMKSKLIKENESKEILSQLLNVQTQLL

SEQ ID NO: 10 - protein, 267 aa, Plasmodium ovale
AQDKDDNILNEITNEYEVVYVKPLAGVYKTLKKQLEAHVTAFHSNVTNMLESRLKKRNYFLEVLNSDLTQYKHATSDNYVIRDAYKLLDFEKKKKLLSSYKYIKDSVEKDVEIATDGIDYYEKMAALYKTYLESVNAQVDAIDKTGDDATKATNKKFLPFLASINAMYETLLEKVNTYNSQLKSSLNSCQLEKIRVGIVVDKLNDYVMFDEKLEELKSSKEKDLTKLYKDIDTSNIINKLKRSGFVDTDESKKLLSELLDVDSAQLL

SEQ ID NO: 11 - protein, 260 aa, Plasmodium malariae
AETKQDDNILKPITNEYEVLYIKPLAGVYRVLRKQIGDQIDAFNSNLTNALDTRKKKRTYFLDVLNSDLIQFKHATSDSYIIKDPYKLLDVDKKAKLIGSYKYIVSAIEKDITSAENGVEYYDKMTKLYKTQLEAVKSAIAEAQKEGDKKTENEKYIPFLTNMQTLYENLLNKINGNIINLKTLITNCNLEKDAVNITISKLTEYSKFDEKIEMFKNSKNEKDIASSGILDILKQKGLVNKNESTKIISELLGVDSNALL

SEQ ID NO: 12 - protein, 267 aa, Plasmodium knowlesi
AENAQPENIVPEGINEYEVVYIKPLAGMYKSIKKQLENHVAAFNTNITDMLDSRLKKRNYFLDVLDSELNPFKYSSSGEYIIKDPYKLLDLEQKKKLLGSYQYIGASVDKDLITAKDGMEYYNKMGELYKQHLEAVNAQIKEIEASVPGEQSQLNAQKEELKKYLPFLNSIQKEYESLVNMAHTYKENLKKFINNCQIEKKETEIIVKKLEDYTKIDENLEIYKKSKKESDVRSSGLLEKLKNSKLINEEESKKVLSQLLNVQTQML

SEQ ID NO: 13 - protein, 124 aa, Artificial Sequence
  His-tagged p19 from P. falciparum
MSHHHHHHHHSMNLAKTVLSNLLDGNLQGMLNISQHQCVKKQCPENSGCFRHLDEREECKCLLNYKQEGDKCVENPNPTCNENNGGCDADAKCTEEDSGSNGKKITCECTKPDSYPLFDGIFCS

SEQ ID NO: 14 - protein, 4 aa, Artificial Sequence
  p33 C-terminal consensus motif
  misc_feature (2)..(2): Xaa can be any naturally occurring amino acid
SXLL

SEQ ID NO: 15 - protein, 121 aa, Artificial Sequence
  His-tagged p19 from P. vivax
MSHHHHHHHHSMENESKEILSQLLNVQTQLLTMSSEHTCIDTNVPDNAACYRYLDGTEEWRCLLTFKEEGGKCVPASNVTCKDNNGGCAPEAECKMTDSNKIVCKCTKEGSEPLFEGVFCS

SEQ ID NO: 16 - protein, 284 aa, Artificial Sequence
  His-tagged p33 from P. vivax
MSHHHHHHHHSMSDQVTTGEAESEAPEILVPAGISDYDVVYLKPLAGMYKTIKKQLENHVNAFNTNITDMLDSRLKKRNYFLEVLNSDLNPFKYSSSGEYIIKDPYKLLDLEKKKKLIGSYKYIGASIDMDLATANDGVTYYNKMGELYKTHLDGVKTEIKKVEDDIKKQDEELKKLGNVNSQDSKKNEFIAKKAELEKYLPFLNSLQKEYESLVSKVNTYTDNLKKVINNCQLEKKEAEITVKKLQDYNKMDEKLEEYKKSEKKNEVKSSGLLEKLMKSKLIK

SEQ ID NO: 17 - protein, 120 aa, Artificial Sequence
  His-tagged p19 from P. ovale
MSHHHHHHHHSMDESKKLLSELLDVDSAQLLSMGSKHKCIDITYPDNAGCYRFSDGREEWRCLLNFKKVGETCVPNNNPTCAENNGGCDPTADCAESENNKITCTCTGQNESFFEGVFCG

SEQ ID NO: 18 - protein, 121 aa, Artificial Sequence
  His-tagged p19 from P. malariae
MSHHHHHHHHSMNESTKIISELLGVDSNALLNISAKHACTETKYPENAGCYRYEDGKEVWRCLLNYKLVDGGCVEDEEPSCQVNNGGCAPEANCTKGDDNKIVCACNAPYSEPIFEGVFCG

SEQ ID NO: 19 - protein, 120 aa, Artificial Sequence
  His-tagged p19 from P. knowlesi
MSHHHHHHHHSMEEESKKVLSQLLNVQTQMLNMSSAHKCIDTNVPENAACYRYLDGTEEWRCLLGFKEVGGKCVPASITCEENNGGCAPEAECTMDDKKEVECKCTKEGFEPLFEGVFCS

SEQ ID NO: 20 - protein, 18 aa, Artificial Sequence
  delta-p33 from P. vivax
NESKEILSQLLNVQTQLL

SEQ ID NO: 21 - protein, 108 aa, Artificial Sequence
  delta-p33-p19 from P. vivax
NESKEILSQLLNVQTQLLTMSSEHTCIDTNVPDNAACYRYLDGTEEWRCLLTFKEEGGKCVPASNVTCKDNNGGCAPEAECKMTDSNKIVCKCTKEGSEPLFEGVFCS

SEQ ID NO: 22 - protein, 19 aa, Artificial Sequence
  delta-p33 from P. falciparum
NLAKTVLSNLLDGNLQGML

SEQ ID NO: 23 - protein, 112 aa, Artificial Sequence
  delta-p33-p19 from P. falciparum
NLAKTVLSNLLDGNLQGMLNISQHQCVKKQCPENSGCFRHLDEREECKCLLNYKQEGDKCVENPNPTCNENNGGCDADAKCTEEDSGSNGKKITCECTKPDSYPLFDGIFCS

SEQ ID NO: 24 - protein, 19 aa, Artificial Sequence
  delta-p33 from P. ovale
DESKKLLSELLDVDSAQLL

SEQ ID NO: 25 - protein, 108 aa, Artificial Sequence
  delta-p33-p19 from P. ovale
DESKKLLSELLDVDSAQLLSMGSKHKCIDITYPDNAGCYRFSDGREEWRCLLNFKKVGETCVPNNNPTCAENNGGCDPTADCAESENNKITCTCTGQNESFFEGVFCG

SEQ ID NO: 26 - protein, 19 aa, Artificial Sequence
  delta-p33 from P. malariae
NESTKIISELLGVDSNALL

SEQ ID NO: 27 - protein, 109 aa, Artificial Sequence
  delta-p33-p19 from P. malariae
NESTKIISELLGVDSNALLNISAKHACTETKYPENAGCYRYEDGKEVWRCLLNYKLVDGGCVEDEEPSCQVNNGGCAPEANCTKGDDNKIVCACNAPYSEPIFEGVFCG

SEQ ID NO: 28 - protein, 19 aa, Artificial Sequence
  delta-p33 from P. knowlesi
EEESKKVLSQLLNVQTQML

SEQ ID NO: 29 - protein, 108 aa, Artificial Sequence
  delta-p33-p19 from P. knowlesi
EEESKKVLSQLLNVQTQMLNMSSAHKCIDTNVPENAACYRYLDGTEEWRCLLGFKEVGGKCVPASITCEENNGGCAPEAECTMDDKKEVECKCTKEGFEPLFEGVFCS

SEQ ID NO: 30 - protein, 834 aa, Artificial Sequence
  Purified fusion polypeptide, N-terminally His tagged
MSHHHHHHHHSMSDQVTTGEAESEAPEILVPAGISDYDVVYLKPLAGMYKTIKKQLENHVNAFNTNITDMLDSRLKKRNYFLEVLNSDLNPFKYSSSGEYIIKDPYKLLDLEKKKKLIGSYKYIGASIDMDLATANDGVTYYNKMGELYKTHLDGVKTEIKKVEDDIKKQDEELKKLGNVNSQDSKKNEFIAKKAELEKYLPFLNSLQKEYESLVSKVNTYTDNLKKVINNCQLEKKEAEITVKKLQDYNKMDEKLEEYKKSEKKNEVKSSGLLEKLMKSKLIKENESKEILSQLLNVQTQLLTMSSEHTCIDTNVPDNAACYRYLDGTEEWRCLLTFKEEGGKCVPASNVTCKDNNGGCAPEAECKMTDSNKIVCKCTKEGSEPLFEGVFCSNLAKTVLSNLLDGNLQGMLNISQHQCVKKQCPENSGCFRHLDEREECKCLLNYKQEGDKCVENPNPTCNENNGGCDADAKCTEEDSGSNGKKITCECTKPDSYPLFDGIFCSDESKKLLSELLDVDSAQLLSMGSKHKCIDITYPDNAGCYRFSDGREEWRCLLNFKKVGETCVPNNNPTCAENNGGCDPTADCAESENNKITCTCTGQNESFFEGVFCGNESTKIISELLGVDSNALLNISAKHACTETKYPENAGCYRYEDGKEVWRCLLNYKLVDGGCVEDEEPSCQVNNGGCAPEANCTKGDDNKIVCACNAPYSEPIFEGVFCGEEESKKVLSQLLNVQTQMLNMSSAHKCIDTNVPENAACYRYLDGTEEWRCLLGFKEVGGKCVPASITCEENNGGCAPEAECTMDDKKEVECKCTKEGFEPLFEGVFCSTMEG

SEQ ID NO: 31 - protein, 832 aa, Artificial Sequence
  His-MSP-multi-His_a
MSHHHHHHHHSMSDQVTTGEAESEAPEILVPAGISDYDVVYLKPLAGMYKTIKKQLENHVNAFNTNITDMLDSRLKKRNYFLEVLNSDLNPFKYSSSGEYIIKDPYKLLDLEKKKKLIGSYKYIGASIDMDLATANDGVTYYNKMGELYKTHLDGVKTEIKKVEDDIKKQDEELKKLGNVNSQDSKKNEFIAKKAELEKYLPFLNSLQKEYESLVSKVNTYTDNLKKVINNCQLEKKEAEITVKKLQDYNKMDEKLEEYKKSEKKNEVKSSGLLEKLMKSKLIKENESKEILSQLLNVQTQLLAMEEESKKVLSQLLNVQTQMLNMSSAHKCIDTNVPENAACYRYLDGTEEWRCLLGFKEVGGKCVPASITCEENNGGCAPEAECTMDDKKEVECKCTKEGFEPLFEGVFCSTMSSEHTCIDTNVPDNAACYRYLDGTEEWRCLLTFKEEGGKCVPASNVTCKDNNGGCAPEAECKMTDSNKIVCKCTKEGSEPLFEGVFCSNLAKTVLSNLLDGNLQGMLNISQHQCVKKQCPENSGCFRHLDEREECKCLLNYKQEGDKCVENPNPTCNENNGGCDADAKCTEEDSGSNGKKITCECTKPDSYPLFDGIFCSDESKKLLSELLDVDSAQLLSMGSKHKCIDITYPDNAGCYRFSDGREEWRCLLNFKKVGETCVPNNNPTCAENNGGCDPTADCAESENNKITCTCTGQNESFFEGVFCGNESTKIISELLGVDSNALLNISAKHACTETKYPENAGCYRYEDGKEVWRCLLNYKLVDGGCVEDEEPSCQVNNGGCAPEANCTKGDDNKIVCACNAPYSEPIFEGVFCG

SEQ ID NO: 32 - protein, 832 aa, Artificial Sequence
  His-MSP-multi-His_b
MSHHHHHHHHSMSDQVTTGEAESEAPEILVPAGISDYDVVYLKPLAGMYKTIKKQLENHVNAFNTNITDMLDSRLKKRNYFLEVLNSDLNPFKYSSSGEYIIKDPYKLLDLEKKKKLIGSYKYIGASIDMDLATANDGVTYYNKMGELYKTHLDGVKTEIKKVEDDIKKQDEELKKLGNVNSQDSKKNEFIAKKAELEKYLPFLNSLQKEYESLVSKVNTYTDNLKKVINNCQLEKKEAEITVKKLQDYNKMDEKLEEYKKSEKKNEVKSSGLLEKLMKSKLIKENESKEILSQLLNVQTQLLAMNESTKIISELLGVDSNALLNISAKHACTETKYPENAGCYRYEDGKEVWRCLLNYKLVDGGCVEDEEPSCQVNNGGCAPEANCTKGDDNKIVCACNAPYSEPIFEGVFCGEEESKKVLSQLLNVQTQMLNMSSAHKCIDTNVPENAACYRYLDGTEEWRCLLGFKEVGGKCVPASITCEENNGGCAPEAECTMDDKKEVECKCTKEGFEPLFEGVFCSTMSSEHTCIDTNVPDNAACYRYLDGTEEWRCLLTFKEEGGKCVPASNVTCKDNNGGCAPEAECKMTDSNKIVCKCTKEGSEPLFEGVFCSNLAKTVLSNLLDGNLQGMLNISQHQCVKKQCPENSGCFRHLDEREECKCLLNYKQEGDKCVENPNPTCNENNGGCDADAKCTEEDSGSNGKKITCECTKPDSYPLFDGIFCSDESKKLLSELLDVDSAQLLSMGSKHKCIDITYPDNAGCYRFSDGREEWRCLLNFKKVGETCVPNNNPTCAENNGGCDPTADCAESENNKITCTCTGQNESFFEGVFCG

SEQ ID NO: 33 - protein, 832 aa, Artificial Sequence
  His-MSP-multi-His_c
MSHHHHHHHHSMSDQVTTGEAESEAPEILVPAGISDYDVVYLKPLAGMYKTIKKQLENHVNAFNTNITDMLDSRLKKRNYFLEVLNSDLNPFKYSSSGEYIIKDPYKLLDLEKKKKLIGSYKYIGASIDMDLATANDGVTYYNKMGELYKTHLDGVKTEIKKVEDDIKKQDEELKKLGNVNSQDSKKNEFIAKKAELEKYLPFLNSLQKEYESLVSKVNTYTDNLKKVINNCQLEKKEAEITVKKLQDYNKMDEKLEEYKKSEKKNEVKSSGLLEKLMKSKLIKENESKEILSQLLNVQTQLLAMDESKKLLSELLDVDSAQLLSMGSKHKCIDITYPDNAGCYRFSDGREEWRCLLNFKKVGETCVPNNNPTCAENNGGCDPTADCAESENNKITCTCTGQNESFFEGVFCGNESTKIISELLGVDSNALLNISAKHACTETKYPENAGCYRYEDGKEVWRCLLNYKLVDGGCVEDEEPSCQVNNGGCAPEANCTKGDDNKIVCACNAPYSEPIFEGVFCGEEESKKVLSQLLNVQTQMLNMSSAHKCIDTNVPENAACYRYLDGTEEWRCLLGFKEVGGKCVPASITCEENNGGCAPEAECTMDDKKEVECKCTKEGFEPLFEGVFCSTMSSEHTCIDTNVPDNAACYRYLDGTEEWRCLLTFKEEGGKCVPASNVTCKDNNGGCAPEAECKMTDSNKIVCKCTKEGSEPLFEGVFCSNLAKTVLSNLLDGNLQGMLNISQHQCVKKQCPENSGCFRHLDEREECKCLLNYKQEGDKCVENPNPTCNENNGGCDADAKCTEEDSGSNGKKITCECTKPDSYPLFDGIFCS

SEQ ID NO: 34 - protein, 832 aa, Artificial Sequence
  His-MSP-multi-His_d
MSHHHHHHHHSMSDQVTTGEAESEAPEILVPAGISDYDVVYLKPLAGMYKTIKKQLENHVNAFNTNITDMLDSRLKKRNYFLEVLNSDLNPFKYSSSGEYIIKDPYKLLDLEKKKKLIGSYKYIGASIDMDLATANDGVTYYNKMGELYKTHLDGVKTEIKKVEDDIKKQDEELKKLGNVNSQDSKKNEFIAKKAELEKYLPFLNSLQKEYESLVSKVNTYTDNLKKVINNCQLEKKEAEITVKKLQDYNKMDEKLEEYKKSEKKNEVKSSGLLEKLMKSKLIKENESKEILSQLLNVQTQLLAMNLAKTVLSNLLDGNLQGMLNISQHQCVKKQCPENSGCFRHLDEREECKCLLNYKQEGDKCVENPNPTCNENNGGCDADAKCTEEDSGSNGKKITCECTKPDSYPLFDGIFCSDESKKLLSELLDVDSAQLLSMGSKHKCIDITYPDNAGCYRFSDGREEWRCLLNFKKVGETCVPNNNPTCAENNGGCDPTADCAESENNKITCTCTGQNESFFEGVFCGNESTKIISELLGVDSNALLNISAKHACTETKYPENAGCYRYEDGKEVWRCLLNYKLVDGGCVEDEEPSCQVNNGGCAPEANCTKGDDNKIVCACNAPYSEPIFEGVFCGEEESKKVLSQLLNVQTQMLNMSSAHKCIDTNVPENAACYRYLDGTEEWRCLLGFKEVGGKCVPASITCEENNGGCAPEAECTMDDKKEVECKCTKEGFEPLFEGVFCSTMSSEHTCIDTNVPDNAACYRYLDGTEEWRCLLTFKEEGGKCVPASNVTCKDNNGGCAPEAECKMTDSNKIVCKCTKEGSEPLFEGVFCS